European Patent Application EP 4 806 914 A1, published September 16, 2026. Title: ＡＡＶのフルカプシドに対するアフィニティポリペプチド. Applicant: Daicel Corporation. Application JP. The sequence listing filed with the application follows.

SEQUENCE LISTING (60 sequences)

SEQ ID NO: 1 - protein, 8 aa, Oryctolagus cuniculus
GFSFSSYG

SEQ ID NO: 2 - protein, 9 aa, Oryctolagus cuniculus
IYGGSSGST

SEQ ID NO: 3 - protein, 13 aa, Oryctolagus cuniculus
ARDRVGGNGYADL

SEQ ID NO: 4 - protein, 6 aa, Oryctolagus cuniculus
QSISSY

SEQ ID NO: 5 - protein, 12 aa, Oryctolagus cuniculus
QSHYDIRNYGVA

SEQ ID NO: 6 - protein, 9 aa, Oryctolagus cuniculus
GFSFSSNYW

SEQ ID NO: 7 - protein, 9 aa, Oryctolagus cuniculus
IYGGSSGST

SEQ ID NO: 8 - protein, 12 aa, Oryctolagus cuniculus
ATVDNGYSDLKL

SEQ ID NO: 9 - protein, 6 aa, Oryctolagus cuniculus
QSIRNW

SEQ ID NO: 10 - protein, 12 aa, Oryctolagus cuniculus
QSSFYADSGEPA

SEQ ID NO: 11 - protein, 9 aa, Oryctolagus cuniculus
GIDFSSGYD

SEQ ID NO: 12 - protein, 8 aa, Oryctolagus cuniculus
IYTGGDSA

SEQ ID NO: 13 - protein, 11 aa, Oryctolagus cuniculus
ANDLDSGTVSI

SEQ ID NO: 14 - protein, 6 aa, Oryctolagus cuniculus
QSISSW

SEQ ID NO: 15 - protein, 12 aa, Oryctolagus cuniculus
AGWTSSTTDGTA

SEQ ID NO: 16 - protein, 9 aa, Oryctolagus cuniculus
GFSFSSSAY

SEQ ID NO: 17 - protein, 9 aa, Oryctolagus cuniculus
MHTISSVDT

SEQ ID NO: 18 - protein, 16 aa, Oryctolagus cuniculus
ARDDRNGYGYPYSFDI

SEQ ID NO: 19 - protein, 6 aa, Oryctolagus cuniculus
QTISSY

SEQ ID NO: 20 - protein, 9 aa, Oryctolagus cuniculus
LTYYGNSHN

SEQ ID NO: 21 - protein, 119 aa, Oryctolagus cuniculus
QSLEESGGGLVKPGASLTLTCTASGFSFSSYGISWFRQAPGKGLEWIGTIYGGSSGSTYYASWAKGRFTISKTSSTTMTLQMASLTAADTATYFCARDRVGGNGYADLWGPGTLVTVTS

SEQ ID NO: 22 - protein, 110 aa, Oryctolagus cuniculus
ELVMTQTAASVEAAVGGTVTIKCQASQSISSYLAWYQQKPGQRPKLLIYRASTLASGVSSRFKGSGSGTEYTLTISDLECDDAATYYCQSHYDIRNYGVAFGGGTEVDIK

SEQ ID NO: 23 - protein, 119 aa, Oryctolagus cuniculus
QSLEESGGDLVKPGASLTLTCTASGFSFSSNYWMFWVRQAPGKGLEWIAHIYGGSSGSTYYASWAKGRFTISKTSSTTVTLQMTSLTAADTATYFCATVDNGYSDLKLWGPGTLVTVTS

SEQ ID NO: 24 - protein, 110 aa, Oryctolagus cuniculus
ELVLTQTADSVEAGVGGTVTIKCQASQSIRNWLSWYQQKPGQPPKLLISRASTLASGVPSRFSGSGSGTEFTLTISDLECDDGATYYCQSSFYADSGEPAFGGGTEVDIK

SEQ ID NO: 25 - protein, 117 aa, Oryctolagus cuniculus
QSVEESGGDLVKPGASLTLTCTASGIDFSSGYDMCWVRQAPGKGLEWIGCIYTGGDSAWYASWAKGRFTISKTSSTTVTLQMTSLTGADTATYFCANDLDSGTVSIWGPGTLVTVTS

SEQ ID NO: 26 - protein, 109 aa, Oryctolagus cuniculus
ELVLTQTAASVSEPVGGTVTIKCQASQSISSWLSWYQQKPGQPPKLLIYQASKLASGVPSRFKGSGSGTQFTLTISDVVCDDAATYYCAGWTSSTTDGTAFGGGTEVVI

SEQ ID NO: 27 - protein, 123 aa, Oryctolagus cuniculus
QSLEESGGDLVKPGASLTLTCTASGFSFSSSAYMCWVRQAPGKGLEWIGCMHTISSVDTYYASWAKGRFAISKASSTTVTLQMTSLTAADTATYFCARDDRNGYGYPYSFDIWGPGTLVTVTS

SEQ ID NO: 28 - protein, 107 aa, Oryctolagus cuniculus
ELDLTQTAASVEAAVGGTITIKCQASQTISSYLAWYQQKPGQPPKLLIYRASTLASGVSSRFKGSGSGTEYTLTISDLECADAATYYCLTYYGNSHNFGGGTEVVIK

SEQ ID NO: 29 - DNA, 24 bp, Oryctolagus cuniculus
  source 1..24: mol_type = other DNA
ggattctccttcagtagctatggc

SEQ ID NO: 30 - DNA, 27 bp, Oryctolagus cuniculus
  source 1..27: mol_type = other DNA
atttatggtggtagtagtggtagcact

SEQ ID NO: 31 - DNA, 39 bp, Oryctolagus cuniculus
  source 1..39: mol_type = other DNA
gcgagagatcgtgttggtggtaatggttatgctgacttg

SEQ ID NO: 32 - DNA, 18 bp, Oryctolagus cuniculus
  source 1..18: mol_type = other DNA
cagagcattagtagctac

SEQ ID NO: 33 - DNA, 36 bp, Oryctolagus cuniculus
  source 1..36: mol_type = other DNA
caaagtcattatgatattaggaattatggtgttgct

SEQ ID NO: 34 - DNA, 27 bp, Oryctolagus cuniculus
  source 1..27: mol_type = other DNA
ggattctccttcagtagcaactactgg

SEQ ID NO: 35 - DNA, 27 bp, Oryctolagus cuniculus
  source 1..27: mol_type = other DNA
atttatggtggtagtagtggtagcact

SEQ ID NO: 36 - DNA, 36 bp, Oryctolagus cuniculus
  source 1..36: mol_type = other DNA
gcgacagttgataatggttattcagatcttaaattg

SEQ ID NO: 37 - DNA, 18 bp, Oryctolagus cuniculus
  source 1..18: mol_type = other DNA
cagagcattcgcaactgg

SEQ ID NO: 38 - DNA, 36 bp, Oryctolagus cuniculus
  source 1..36: mol_type = other DNA
caaagttctttttatgccgatagtggggagcctgct

SEQ ID NO: 39 - DNA, 27 bp, Oryctolagus cuniculus
  source 1..27: mol_type = other DNA
ggaatcgacttcagtagcggctacgac

SEQ ID NO: 40 - DNA, 24 bp, Oryctolagus cuniculus
  source 1..24: mol_type = other DNA
atttatactggtggtgatagcgca

SEQ ID NO: 41 - DNA, 33 bp, Oryctolagus cuniculus
  source 1..33: mol_type = other DNA
gcgaatgatttagactctggtactgtaagcatc

SEQ ID NO: 42 - DNA, 18 bp, Oryctolagus cuniculus
  source 1..18: mol_type = other DNA
cagagcattagcagttgg

SEQ ID NO: 43 - DNA, 36 bp, Oryctolagus cuniculus
  source 1..36: mol_type = other DNA
gcaggatggacaagtagtactactgatggtactgct

SEQ ID NO: 44 - DNA, 27 bp, Oryctolagus cuniculus
  source 1..27: mol_type = other DNA
ggattctccttcagtagcagcgcctac

SEQ ID NO: 45 - DNA, 27 bp, Oryctolagus cuniculus
  source 1..27: mol_type = other DNA
atgcatactattagtagtgttgacact

SEQ ID NO: 46 - DNA, 48 bp, Oryctolagus cuniculus
  source 1..48: mol_type = other DNA
gcgagagatgataggaatggttatggttatccttattcttttgacatc

SEQ ID NO: 47 - DNA, 18 bp, Oryctolagus cuniculus
  source 1..18: mol_type = other DNA
cagaccattagtagttat

SEQ ID NO: 48 - DNA, 27 bp, Oryctolagus cuniculus
  source 1..27: mol_type = other DNA
ctaacctattatggtaatagtcataac

SEQ ID NO: 49 - DNA, 357 bp, Oryctolagus cuniculus
  source 1..357: mol_type = other DNA
cagtcgttggaggagtccgggggaggcctggtcaagcctggggcatccctgacactcacctgcacagcctctggattctccttcagtagctatggcattagctggttccgccaggctccagggaaggggctggagtggatcggaaccatttatggtggtagtagtggtagcacttactacgcgagctgggcgaaaggccgattcaccatctccaaaacctcgtcgaccacgatgactctgcaaatggccagtctgacagccgcggacacggccacctatttctgtgcgagagatcgtgttggtggtaatggttatgctgacttgtggggcccaggcaccctcgtcaccgtcactagt

SEQ ID NO: 50 - DNA, 330 bp, Oryctolagus cuniculus
  source 1..330: mol_type = other DNA
gagctcgtgatgacccagactgcagcctccgtggaggcagctgtgggaggcacagtcaccatcaagtgccaggccagtcagagcattagtagctacttagcctggtatcagcagaaaccagggcagcgtcccaagctcctgatctacagggcatccactctggcatctggggtctcatcgcggttcaaaggcagtggatctgggacagagtacacgctcaccatcagcgacctggagtgtgacgatgctgccacttactactgtcaaagtcattatgatattaggaattatggtgttgctttcggcggagggaccgaggtggacatcaaa

SEQ ID NO: 51 - DNA, 357 bp, Oryctolagus cuniculus
  source 1..357: mol_type = other DNA
cagtcgctggaggagtccgggggagacctggtcaagcctggggcatccctgacactcacctgcacagcctctggattctccttcagtagcaactactggatgttctgggtccgccaggctccagggaaggggctggagtggatcgcacacatttatggtggtagtagtggtagcacttactacgcgagctgggcgaaaggccgattcaccatctccaagacctcgtcgaccacggtgactctgcaaatgaccagtctgacagccgcggacacggccacctatttctgtgcgacagttgataatggttattcagatcttaaattgtggggcccaggcaccctggtcaccgtcactagt

SEQ ID NO: 52 - DNA, 330 bp, Oryctolagus cuniculus
  source 1..330: mol_type = other DNA
gagctcgtgctgacccagactgcagactccgtggaggcaggtgtgggaggcacagtcaccatcaagtgccaggccagtcagagcattcgcaactggttatcctggtatcagcagaaaccagggcagcctcccaagctcctgatctccagggcatccactctggcatctggggtcccctcgcggttcagtggcagtggatctgggacagagttcactctcaccatcagcgacctggagtgtgacgatggtgccacttactactgtgtttcaagaaaaatacggctatcacccctcggacgaaagccgcctccctggctccacctgtagttt

SEQ ID NO: 53 - DNA, 351 bp, Oryctolagus cuniculus
  source 1..351: mol_type = other DNA
cagtcggtggaggagtccgggggagacctggtcaagcctggggcatccctgacactcacctgcacagcctctggaatcgacttcagtagcggctacgacatgtgctgggtccgccaggctccagggaaggggctggagtggatcggatgcatttatactggtggtgatagcgcatggtacgcgagctgggcgaaaggccgattcaccatctccaaaacctcgtcgaccacggtgactctgcaaatgaccagtctgacaggcgcggacacggccacctatttctgtgcgaatgatttagactctggtactgtaagcatctggggcccaggcaccctggtcaccgtcactagt

SEQ ID NO: 54 - DNA, 327 bp, Oryctolagus cuniculus
  source 1..327: mol_type = other DNA
gagctcgtgctgacccagactgcagcctccgtgtctgaacctgtgggaggcacagtcaccatcaagtgccaggccagtcagagcattagcagttggttatcctggtatcagcagaaaccagggcagcctcccaagctcctgatctaccaggcatccaaactggcatctggggtcccatcgcggttcaaaggcagtggatctgggacacagttcactctcaccatcagcgatgtggtgtgtgacgatgctgccacttactactgtgcaggatggacaagtagtactactgatggtactgctttcggcggagggaccgaggtggtcatc

SEQ ID NO: 55 - DNA, 369 bp, Oryctolagus cuniculus
  source 1..369: mol_type = other DNA
cagtcgttggaggagtccgggggagacctggtcaagcctggggcatccctgacactcacctgcacagcctctggattctccttcagtagcagcgcctacatgtgctgggtccgccaggctccagggaaggggctggagtggatcggatgcatgcatactattagtagtgttgacacttactacgcgagctgggcgaaaggccgattcgccatctccaaagcctcgtcgaccacggtgactctgcaaatgaccagtctgacagccgcggacacggccacctatttctgtgcgagagatgataggaatggttatggttatccttattcttttgacatctggggcccaggcaccctcgtcaccgtcactagt

SEQ ID NO: 56 - DNA, 321 bp, Oryctolagus cuniculus
  source 1..321: mol_type = other DNA
gagctcgatctgacccagactgcagcctccgtggaggcagctgtgggaggcacaatcaccatcaagtgccaggccagtcagaccattagtagttatttagcctggtatcagcagaaaccagggcagcctcccaagctcctgatctacagggcatccactctggcatctggggtctcatcaaggttcagaggcagtggatctgggacagaatacactctcaccatcagcgacctggagtgtgccgatgctgccacttactactgtctaacctattatggtaatagtcataacttcggcggagggaccgaggtggtgatcaaa

SEQ ID NO: 57 - protein, 15 aa, synthetic construct
GGGGSGGGGSGGGGS

SEQ ID NO: 58 - protein, 29 aa, synthetic construct
RSAAAGGGSEQKLISEEDLGGGSHHHHHH

SEQ ID NO: 59 - protein, 30 aa, synthetic construct
TGSAAAGGGSEQKLISEEDLGGGSHHHHHH

SEQ ID NO: 60 - protein, 29 aa, synthetic construct
GSAAAGGGSEQKLISEEDLGGGSHHHHHH